European Patent Application EP 4 159 763 A1, published April 5, 2023. Title: Anti CD73 antibody and the use thereof. Applicant: BrightPath Biotherapeutics Co., Ltd. The sequence listing filed with the application follows.

SEQUENCE LISTING (88 sequences)

SEQ ID NO: 1 - protein, 5 aa, Artificial Sequence
  CDR1 of 002 antibody HC
  MISC_FEATURE (2)..(2): Cys or Ser
DXNMD

SEQ ID NO: 2 - protein, 17 aa, Artificial Sequence
  CDR2 of 002 antibody HC
DINPNNGGTIYNQKFKG

SEQ ID NO: 3 - protein, 9 aa, Artificial Sequence
  CDR3 of 002 antibody HC
TNWDYAMDY

SEQ ID NO: 4 - protein, 11 aa, Artificial Sequence
  CDR1 of 002 antibody LC
  MISC_FEATURE (9)..(9): Asn, Asp or Gln
KASQDINSXLS

SEQ ID NO: 5 - protein, 7 aa, Artificial Sequence
  CDR2 of 002 antibody LC
RANRLID

SEQ ID NO: 6 - protein, 9 aa, Artificial Sequence
  CDR3 of 002 antibody LC
  MISC_FEATURE (1)..(1): Leu or Gln
XQYDVFPRT

SEQ ID NO: 7 - protein, 118 aa, Mus musculus
QVQMKQSGPELVKPGASVKIPCKASGYTFTDCNMDWVKQSHGESLEWIGDINPNNGGTIYNQKFKGKVTLTIDKSSSTAYMELRSLTSEDTAVYYCARTNWDYAMDYWGQGTSVTVSS

SEQ ID NO: 8 - protein, 107 aa, Mus musculus
DIQMTQSPSSMYASLGERVTITCKASQDINSNLSWFQQKPGKSPKTLIYRANRLIDGVPSRFSGSGSGQDYSLTISSLEYEDMGIYYCLQYDVFPRTFGGGTKLELK

SEQ ID NO: 9 - protein, 5 aa, Mus musculus
SFGMH

SEQ ID NO: 10 - protein, 17 aa, Mus musculus
YISSGSRTIYYADTVRG

SEQ ID NO: 11 - protein, 12 aa, Mus musculus
DFGSSSPNYFDY

SEQ ID NO: 12 - protein, 15 aa, Mus musculus
RASESVDNYGISFMN

SEQ ID NO: 13 - protein, 7 aa, Mus musculus
AASNQGS

SEQ ID NO: 14 - protein, 9 aa, Mus musculus
QQSKEVPWT

SEQ ID NO: 15 - protein, 121 aa, Mus musculus
DVKLVESGGGLVQPGGSRKLSCAASGFTFSSFGMHWVRQAPEKGLEWVAYISSGSRTIYYADTVRGRFTISRDNSKNTLFLQLTSLRSEDTAIYYCASDFGSSSPNYFDYWGQGTTVTVSS

SEQ ID NO: 16 - protein, 111 aa, Mus musculus
DIVMTQSPASLAVSLGQRATISCRASESVDNYGISFMNWFQQKPGQPPKLLIYAASNQGSGVPARFSGSGSGTDFSLNIHPMEEDDTAMYFCQQSKEVPWTFGGGTRLEIK

SEQ ID NO: 17 - protein, 5 aa, Mus musculus
GYWMN

SEQ ID NO: 18 - protein, 17 aa, Mus musculus
RIDPYDSETHYSQKFKD

SEQ ID NO: 19 - protein, 11 aa, Mus musculus
SSPITTAPFDY

SEQ ID NO: 20 - protein, 15 aa, Mus musculus
RASESVDYYGFSFMN

SEQ ID NO: 21 - protein, 7 aa, Mus musculus
AASTQGS

SEQ ID NO: 22 - protein, 9 aa, Mus musculus
QQSKEVPYT

SEQ ID NO: 23 - protein, 120 aa, Mus musculus
QVQLQQPGAELVRPGTSVKLSCKASGYTFTGYWMNWLKQRPDQGLEWIGRIDPYDSETHYSQKFKDKAILTVHKSSSTAYIQLNSLTSEDSAVYYCTRSSPITTAPFDYWGRGTTLTVSS

SEQ ID NO: 24 - protein, 111 aa, Mus musculus
NIVLTQSPASLAVSLGQRATISCRASESVDYYGFSFMNWFQLKPGQPPKLLIYAASTQGSGVPARFSGSGSGTDFSLNIHPMEEDDIAMYFCQQSKEVPYTFGGGTKLELK

SEQ ID NO: 25 - protein, 5 aa, Mus musculus
SYGVS

SEQ ID NO: 26 - protein, 16 aa, Mus musculus
VIWGDGSTNYHSALIS

SEQ ID NO: 27 - protein, 13 aa, Mus musculus
TNIFYDYDWYLDV

SEQ ID NO: 28 - protein, 16 aa, Mus musculus
RSSQSLVHSNGNTYLH

SEQ ID NO: 29 - protein, 7 aa, Mus musculus
KVSNRFS

SEQ ID NO: 30 - protein, 9 aa, Mus musculus
SHSTHVPWT

SEQ ID NO: 31 - protein, 121 aa, Mus musculus
DVQLVESGPGLVAPSQSLSITCTVSGFSLTSYGVSWVRQPPGKGLEWLGVIWGDGSTNYHSALISRLSISKDNSKSQVFLKLNSLQTDDTATYYCAKTNIFYDYDWYLDVWGAGTTVTVSS

SEQ ID NO: 32 - protein, 112 aa, Mus musculus
DIVMTQAPLSLPVSLGDQASISCRSSQSLVHSNGNTYLHWYLQKPGQSPKLLIYKVSNRFSGVPDRFSGSGSGTDFTLKISRVEAEDLGVYFCSHSTHVPWTFGGGTKLELK

SEQ ID NO: 33 - protein, 5 aa, Mus musculus
SYWMH

SEQ ID NO: 34 - protein, 17 aa, Mus musculus
EINPSNARTNYNENFKS

SEQ ID NO: 35 - protein, 10 aa, Mus musculus
RGTSGNYFDF

SEQ ID NO: 36 - protein, 11 aa, Mus musculus
KASQDINTYLS

SEQ ID NO: 37 - protein, 7 aa, Mus musculus
RANRLVD

SEQ ID NO: 38 - protein, 9 aa, Mus musculus
LQYDEFPYT

SEQ ID NO: 39 - protein, 119 aa, Mus musculus
QVQLQQPGAELVKPGVSVKLSCKASGYTFTSYWMHWVKQRPGQGPEWIGEINPSNARTNYNENFKSKATLTVDKSSTTAYMHFSRLTSEDSAVYYCARRGTSGNYFDFWGQGTTVTVSS

SEQ ID NO: 40 - protein, 107 aa, Mus musculus
DIQMTQSPSSMYASLGERVTITCKASQDINTYLSWFQQKPGKSPKTLIYRANRLVDGVPSRFSGSGSGEDYSLTISSLEYEDMGIYYCLQYDEFPYTFGGGTRLEIK

SEQ ID NO: 41 - protein, 5 aa, Mus musculus
SYWMN

SEQ ID NO: 42 - protein, 17 aa, Mus musculus
KIDPYDSETHYNQKFKD

SEQ ID NO: 43 - protein, 8 aa, Mus musculus
IRYGTFDY

SEQ ID NO: 44 - protein, 11 aa, Mus musculus
KASQDINNYLS

SEQ ID NO: 45 - protein, 7 aa, Mus musculus
RANILVD

SEQ ID NO: 46 - protein, 9 aa, Mus musculus
LQYDEFPYT

SEQ ID NO: 47 - protein, 117 aa, Mus musculus
QVQLQQPGAELVRPGASVKLSCKASGYTFTSYWMNWVKQRPEQGLEWIGKIDPYDSETHYNQKFKDKAILTVDKSSSTAFMQLSSLTSEDSAVYYCARIRYGTFDYWGQGTTLTVSS

SEQ ID NO: 48 - protein, 107 aa, Mus musculus
DIVMTQSPSSMYASLGERVTITCKASQDINNYLSWFQQKPGKSPKTLIYRANILVDGVPSGFSGSGSGQDYSLTISSLEYEDMGIYYCLQYDEFPYTFGGGTRLEIK

SEQ ID NO: 49 - protein, 5 aa, Mus musculus
SYWMH

SEQ ID NO: 50 - protein, 17 aa, Mus musculus
EINPSNGRTNYNEKFKN

SEQ ID NO: 51 - protein, 10 aa, Mus musculus
RGTSGNYFDY

SEQ ID NO: 52 - protein, 11 aa, Mus musculus
KASQDINTYLS

SEQ ID NO: 53 - protein, 7 aa, Mus musculus
RANRLVD

SEQ ID NO: 54 - protein, 9 aa, Mus musculus
LQYDEFPYT

SEQ ID NO: 55 - protein, 119 aa, Mus musculus
QVQLKQSGAELVKPGASVKLSCKASGYTFTSYWMHWVKQRPGQGPEWIGEINPSNGRTNYNEKFKNRATLTVDKSSSTAYMQLSRLTSEDSAVYYCARRGTSGNYFDYWGQGTTLTVSS

SEQ ID NO: 56 - protein, 107 aa, Mus musculus; identical to SEQ ID NO: 40

SEQ ID NO: 57 - protein, 5 aa, Mus musculus
SYWMN

SEQ ID NO: 58 - protein, 17 aa, Mus musculus
RIDPYDSEAHYNQKFKD

SEQ ID NO: 59 - protein, 8 aa, Mus musculus
IRYGTFDY

SEQ ID NO: 60 - protein, 11 aa, Mus musculus
KASQDINSYLS

SEQ ID NO: 61 - protein, 7 aa, Mus musculus
RSNSLVD

SEQ ID NO: 62 - protein, 9 aa, Mus musculus
LQYDEFPYT

SEQ ID NO: 63 - protein, 117 aa, Mus musculus
QVQLQQSGAELVRPGASVKLSCKASGYTFTSYWMNWVKQRPEPGLEWIGRIDPYDSEAHYNQKFKDKAILTVDKSSSTAYMQLSSLTSEDSAVYYCTRIRYGTFDYWGQGTTLTVSS

SEQ ID NO: 64 - protein, 108 aa, Mus musculus
DIVLTQSPSSMYASLGERVTITCKASQDINSYLSWFQQKPGKSPKTLIYRSNSLVDGVPSRFSGSGSGQDYSLTISSLEYEDMGSYYCLQYDEFPYTFGGGTRLEIKR

SEQ ID NO: 65 - protein, 118 aa, Artificial Sequence
  HC variable domain of 002_6_h1 antibody
QVQLVQSGAEVKKPGASVKVSCKASGYTFTDSNMDWVRQAPGQRLEWMGDINPNNGGTIYNQKFKGRVTITRDTSASTAYMELSSLRSEDTAVYYCARTNWDYAMDYWGQGTLVTVSS

SEQ ID NO: 66 - protein, 107 aa, Artificial Sequence
  LC variable domain of 002_6_h1 antibody
DIQMTQSPSSLSASVGDRVTITCKASQDINSQLSWYQQKPGKAPKLLIYRANRLIDGVPSRFSGSGSGTDFTLTISSLQPEDFATYYCQQYDVFPRTFGQGTKLEIK

SEQ ID NO: 67 - protein, 118 aa, Artificial Sequence
  HC variable domain of 002_6_h2 antibody
QVQMKQSGAEVKKPGASVKVSCKASGYTFTDSNMDWVRQAPGQRLEWMGDINPNNGGTIYNQKFKGRVTITIDTSASTAYMELSSLRSEDTAVYYCARTNWDYAMDYWGQGTLVTVSS

SEQ ID NO: 68 - protein, 107 aa, Artificial Sequence
  LC variable domain of 002_6_h2 antibody
DIQMTQSPSSMSASVGDRVTITCKASQDINSQLSWYQQKPGKAPKTLIYRANRLIDGVPSRFSGSGSGTDFTLTISSLQYEDMATYYCLQYDVFPRTFGQGTKLEIK

SEQ ID NO: 69 - protein, 118 aa, Artificial Sequence
  HC variable domain of 002_6_h3 antibody
QVQLLQSAAEVRKPGASVKVSCKASGYTFTDSNMDWVRQAPGQGLEWMGDINPNNGGTIYNQKFKGRVTMTTDTSRRTAYMELRSLRSDDTAVYYCARTNWDYAMDYWGQGTTVTVSS

SEQ ID NO: 70 - protein, 107 aa, Artificial Sequence
  LC variable domain of 002_6_h3 antibody
DIQMTQSPSFLSASVGDRVTITCKASQDINSQLSWYQQKPGKAPKLLIYRANRLIDGVPSRFSGSGSGTEFTLTISSLQPEDFATYYCQQYDVFPRTFGGGTKLEIK

SEQ ID NO: 71 - protein, 118 aa, Artificial Sequence
  HC variable domain of 002_6_h4 antibody
QVQMKQSAAEVRKPGASVKVSCKASGYTFTDSNMDWVRQAPGQGLEWMGDINPNNGGTIYNQKFKGRVTMTIDTSRSTAYMELRSLRSDDTAVYYCARTNWDYAMDYWGQGTTVTVSS

SEQ ID NO: 72 - protein, 107 aa, Artificial Sequence
  LC variable domain of 002_6_h4 antibody
DIQMTQSPSFLSASVGDRVTITCKASQDINSQLSWYQQKPGKAPKTLIYRANRLIDGVPSRFSGSGSGTDFTLTISSLQYEDMATYYCLQYDVFPRTFGGGTKLEIK

SEQ ID NO: 73 - protein, 118 aa, Artificial Sequence
  HC variable domain of 002_6_h5 antibody
QVQLQESGAEVKKPGASVKVSCKASGYTFTDSNMDWVRQAPGQGLEWMGDINPNNGGTIYNQKFKGRVTMTRDTSTSTVYMELSSLRSEDTAVYYCARTNWDYAMDYWGQGTLVTVSS

SEQ ID NO: 74 - protein, 107 aa, Artificial Sequence
  LC variable domain of 002_6_h5 antibody
DIQVTQSPSFLSASVGDRVTITCKASQDINSQLSWYQQKPGKAPKLLIYRANRLIDGVPSRFSGSGSGTEFTLTISSLQPEDFATYYCQQYDVFPRTFGGGTKVEIK

SEQ ID NO: 75 - protein, 118 aa, Artificial Sequence
  HC variable domain of 002_6_h6 antibody
QVQMKESGAEVKKPGASVKVSCKASGYTFTDSNMDWVRQAPGQGLEWMGDINPNNGGTIYNQKFKGRVTMTIDTSTSTVYMELSSLRSEDTAVYYCARTNWDYAMDYWGQGTLVTVSS

SEQ ID NO: 76 - protein, 107 aa, Artificial Sequence
  LC variable domain of 002_6_h6 antibody
DIQVTQSPSFLSASVGDRVTITCKASQDINSQLSWYQQKPGKAPKTLIYRANRLIDGVPSRFSGSGSGTDFTLTISSLQYEDMATYYCLQYDVFPRTFGGGTKVEIK

SEQ ID NO: 77 - protein, 118 aa, Artificial Sequence
  HC variable domain of 002_6_h7 antibody
EVQLVESGAEVKKPGASVKVSCKASGYTFTDSNMDWVRQAPGQGLEWMGDINPNNGGTIYNQKFKGRVTMTRDTSINTAYMELSRLRSDDTAVYYCAMTNWDYAMDYWGQGTTVTVSS

SEQ ID NO: 78 - protein, 107 aa, Artificial Sequence
  LC variable domain of 002_6_h7 antibody
DIVMTQSPSSLSASVGDRVTITCKASQDINSQLSWYQQKPGKAPKLLIYRANRLIDGVPSRFSGSGSGTDFTLTISSLQPEDFATYYCQQYDVFPRTFGQGTKVEIK

SEQ ID NO: 79 - protein, 118 aa, Artificial Sequence; identical to SEQ ID NO: 77
  HC variable domain of 002_6_h8 antibody

SEQ ID NO: 80 - protein, 107 aa, Artificial Sequence; identical to SEQ ID NO: 78
  LC variable domain of 002_6_h8 antibody

SEQ ID NO: 81 - protein, 120 aa, Artificial Sequence
  HC variable domain of 004_h3 antibody
EVQLVQSGAEVKKPGESLKISCKASGYTFTGYWMNWLRQMPDKGLEWMGRIDPYDSETHYSQKFKDKVTITAHKSSSTAYLQWSSLKASDSAIYYCARSSPITTAPFDYWGQGTTVTVSS

SEQ ID NO: 82 - protein, 111 aa, Artificial Sequence
  LC variable domain of 004_h3 antibody
DIVMTQSPASLAVSLGERATISCRASESVDYYGFSFMNWYQQKPGQPPKLLIYAASTQGSGVPDRFSGSGSGTDFTLTISSLQAEDVAVYYCQQSKEVPYTFGGGTKVEIK

SEQ ID NO: 83 - protein, 119 aa, Artificial Sequence
  HC variable domain of 006_hKB antibody
QVQLLQSGAEVKKPGESVKISCKASGYTFTSYWMHWVKQRPGQGLEWIGEINPSNARTNYNENFKSRFTITVDKSTSTAYMQFSRLRSDDTAVYYCARRGTSGNYFDFWGQGTMLTVSS

SEQ ID NO: 84 - protein, 107 aa, Artificial Sequence
  LC variable domain of 006_hKB antibody
DIQMTQSPSSLSASLGQRVTITCKASQDINTYLSWFQQKPGKPPKTLIYRANRLVDGVPSRFSGSGSGEDYSLTISSLQSEDFGVYYCLQYDEFPYTFGPGTRLEIK

SEQ ID NO: 85 - protein, 117 aa, Artificial Sequence
  HC variable domain of 007_h1 antibody
QVQLVQSGAEVKKPGASVKVSCKASGYTFTSYWMNWVRQAPGQRLEWMGKIDPYDSETHYNQKFKDRVTITVDTSSSTAYMELSSLRSEDTAVYYCARIRYGTFDYWGQGTLVTVSS

SEQ ID NO: 86 - protein, 107 aa, Artificial Sequence
  LC variable domain of 007_h1 antibody
DIQMTQSPSSLSASVGDRVTITCKASQDINNYLSWYQQKPGKAPKTLIYRANILVDGVPSGFSGSGSGTDFTLTISSLQYEDMATYYCLQYDEFPYTFGQGTKLEIK

SEQ ID NO: 87 - protein, 119 aa, Artificial Sequence
  HC variable domain of 008_h4 antibody
QVQLVQSGAEVKKPGASVKVSCKASGYTFTSYWMHWVRQRPGQGLEWMGEINPSNGRTNYNEKFKNRATITADKSSSTAYMELSSLRSEDTAVYYCARRGTSGNYFDYWGQGTLVTVSS

SEQ ID NO: 88 - protein, 107 aa, Artificial Sequence
  LC variable domain of 008_h4 antibody
DIQMTQSPSSLSASVGDRVTITCKASQDINTYLSWFQQKPGKAPKTLIYRANRLVDGVPSRFSGSGYGTDFTLTISSLQYEDMATYYCLQYDEFPYTFGGGTKVEIK